European Patent Application EP 4 570 823 A1, published June 18, 2025. Title: IMPROVED ANTIBODY SPECIFICALLY BINDING TO AMYLOID-β OLIGOMERS. Applicant: Shen Zhen Wisdom Biopharm Co., Ltd. The sequence listing filed with the application follows.

SEQUENCE LISTING (36 sequences)

SEQ ID NO: 1 - protein, 242 aa, synthetic construct
MAEVQLLESGGGLVQPGGSLRLSCAASGFTFSSYAMSWVRQAPGKGLEWVSGISNLGLTTGYADSVKGRFTISRDNSKNTLYLQMNSLRAEDTAVYYCAKTTSRFDYWGQGTLVTVSSGGGGSGGGGSGGGGSTDIQMTQSPSSLSASVGDRVTITCRASQSISSYLNWYQQKPGKAPKLLIYKASYLQSGVPSRFSGSGSGTDFTLTISSLQPEDFATYYCQQTHRPPVTFGQGTKVEIKR

SEQ ID NO: 2 - DNA, 17 bp, synthetic construct
  source 1..17: mol_type = other DNA
caggaaacagctatgac

SEQ ID NO: 3 - DNA, 17 bp, synthetic construct
  source 1..17: mol_type = other DNA
ctatgcggccccattca

SEQ ID NO: 4 - protein, 242 aa, synthetic construct
MAEVQLLESGGGLVQPGGSLRLSCAASGFTFSSYAMSWVRQAPGKGLEWVSGISNLGLTTGYADSVKGRFTISRDNSKNTLYLQMNSLRAEDTAVYYCAKTTSRFDYWGQGTLVTVSSGGGGSGGGGSGGGGSTDIQMTQSPSSLSASVGDRVTITCRASQSISSYLNWYQQKPGKAPKLLIYKASYLQSGVPSRFSGSGSGTDFTLTISSLQPEDFATYYCQQSNFRPVTFGQGTKVEIKR

SEQ ID NO: 5 - protein, 242 aa, synthetic construct
MAEVQLLESGGGLVQPGGSLRLSCAASGFTFSSYAMSWVRQAPGKGLEWVSGISNLGLTTGYADSVKGRFTISRDNSKNTLYLQMNSLRAEDTAVYYCAKTTSRFDYWGQGTLVTVSSGGGGSGGGGSGGGGSTDIQMTQSPSSLSASVGDRVTITCRASQSISSYLNWYQQKPGKAPKLLIYKASYLQSGVPSRFSGSGSGTDFTLTISSLQPEDFATYYCQNSAVRPVTFGQGTKVEIKR

SEQ ID NO: 6 - protein, 242 aa, synthetic construct
MAEVQLLESGGGLVQPGGSLRLSCAASGFTFSSYAMSWVRQAPGKGLEWVSGISNLGLTTGYADSVKGRFTISRDNSKNTLYLQMNSLRAEDTAVYYCAKTTSRFDYWGQGTLVTVSSGGGGSGGGGSGGGGSTDIQMTQSPSSLSASVGDRVTITCRASQSISSYLNWYQQKPGKAPKLLIYKASYLQSGVPSRFSGSGSGTDFTLTISSLQPEDFATYYCQNSFERPVTFGQGTKVEIKR

SEQ ID NO: 7 - protein, 242 aa, synthetic construct
MAEVQLLESGGGLVQPGGSLRLSCAASGFTFSSYAMSWVRQAPGKGLEWVSGISNLGLTTGYADSVKGRFTISRDNSKNTLYLQMNSLRAEDTAVYYCAKTTSRFDYWGQGTLVTVSSGGGGSGGGGSGGGGSTDIQMTQSPSSLSASVGDRVTITCRASQSISSYLNWYQQKPGKAPKLLIYKASYLQSGVPSRFSGSGSGTDFTLTISSLQPEDFATYYCQQAWVRPVTFGQGTKVEIKR

SEQ ID NO: 8 - protein, 242 aa, synthetic construct
MAEVQLLESGGGLVQPGGSLRLSCAASGFTFSSYAMSWVRQAPGKGLEWVSGISNLGLTTGYADSVKGRFTISRDNSKNTLYLQMNSLRAEDTAVYYCAKTTSRFDYWGQGTLVTVSSGGGGSGGGGSGGGGSTDIQMTQSPSSLSASVGDRVTITCRASQSISSYLNWYQQKPGKAPKLLIYKASYLQSGVPSRFSGSGSGTDFTLTISSLQPEDFATYYCQQSGSRPVTFGQGTKVEIKR

SEQ ID NO: 9 - protein, 242 aa, synthetic construct
MAEVQLLESGGGLVQPGGSLRLSCAASGFTFSSYAMSWVRQAPGKGLEWVSGISNLGLTTGYADSVKGRFTISRDNSKNTLYLQMNSLRAEDTAVYYCAKTTSRFDYWGQGTLVTVSSGGGGSGGGGSGGGGSTDIQMTQSPSSLSASVGDRVTITCRASQSISSYLNWYQQKPGKAPKLLIYKASYLQSGVPSRFSGSGSGTDFTLTISSLQPEDFATYYCQQRVRRPVTFGQGTKVEIKR

SEQ ID NO: 10 - protein, 5 aa, synthetic construct
SYAMS

SEQ ID NO: 11 - protein, 17 aa, synthetic construct
GISNLGLTTGYADSVKG

SEQ ID NO: 12 - protein, 7 aa, synthetic construct
TTSRFDY

SEQ ID NO: 13 - protein, 11 aa, synthetic construct
RASQSISSYLN

SEQ ID NO: 14 - protein, 7 aa, synthetic construct
KASYLQS

SEQ ID NO: 15 - protein, 9 aa, synthetic construct
QNSAVRPVT

SEQ ID NO: 16 - protein, 9 aa, synthetic construct
  SITE 2: note = X224 may be N or Q
  SITE 3: note = X225 may be S or T
  SITE 4: note = X226 may be a non-polar, hydrophobic amino acid having similar properties to those of alanine
  SITE 5: note = X227 may be a hydrophobic amino acid having similar properties to those of valine
  SITE 6: note = X228 may be an aliphatic amino acid having a similar structure to that of arginine
QXXXXXPVT

SEQ ID NO: 17 - protein, 214 aa, synthetic construct
DIQMTQSPSSLSASVGDRVTITCRASQSISSYLNWYQQKPGKAPKLLIYKASYLQSGVPSRFSGSGSGTDFTLTISSLQPEDFATYYCQNSAVRPVTFGQGTKVEIKRTVAAPSVFIFPPSDEQLKSGTASVVCLLNNFYPREAKVQWKVDNALQSGNSQESVTEQDSKDSTYSLSSTLTLSKADYEKHKVYACEVTHQGLSSPVTKSFNRGEC

SEQ ID NO: 18 - protein, 443 aa, synthetic construct
EVQLLESGGGLVQPGGSLRLSCAASGFTFSSYAMSWVRQAPGKGLEWVSGISNLGLTTGYADSVKGRFTISRDNSKNTLYLQMNSLRAEDTAVYYCAKTTSRFDYWGQGTLVTVSSASTKGPSVFPLAPCSRSTSESTAALGCLVKDYFPEPVTVSWNSGALTSGVHTFPAVLQSSGLYSLSSVVTVPSSSLGTKTYTCNVDHKPSNTKVDKRVESKYGPPCPPCPAPEFEGGPSVFLFPPKPKDTLYITREPEVTCVVVDVSQEDPEVQFNWYVDGVEVHNAKTKPREEQFNSTYRVVSVLTVLHQDWLNGKEYKCKVSNKGLGSSIEKTISKAKGQPREPQVYTLPPSQEEMTKNQVSLTCLVKGFYPSDIAVEWESNGQPENNYKTTPPVLDSDGSFFLYSRLTVDKSRWQEGNVFSCSVMHEALHNHYTQKSLSLSLGK

SEQ ID NO: 19 - protein, 443 aa, synthetic construct
EVQLLESGGGLVQPGGSLRLSCAASGFTFSSYAMSWVRQAPGKGLEWVSGISNLGLTTGYADSVKGRFTISRDNSKNTLYLQMNSLRAEDTAVYYCAKTTSRFDYWGQGTLVTVSSASTKGPSVFPLAPCSRSTSESTAALGCLVKDYFPEPVTVSWNSGALTSGVHTFPAVLQSSGLYSLSSVVTVPSSSLGTKTYTCNVDHKPSNTKVDKRVESKYGPPCPPCPAPEAEGGPSVFLFPPKPKDTLYITREPEVTCVVVDVSQEDPEVQFNWYVDGVEVHNAKTKPREEQFNSTYRVVSVLTVLHQDWLNGKEYKCKVSNKGLPSSIEKTISKAKGQPREPQVYTLPPSQEEMTKNQVSLTCLVKGFYPSDIAVEWESNGQPENNYKTTPPVLDSDGSFFLYSKLTVDKSRWQEGNVFSCSVMHEALHNHYTQKSLSLSLGK

SEQ ID NO: 20 - protein, 443 aa, synthetic construct
EVQLLESGGGLVQPGGSLRLSCAASGFTFSSYAMSWVRQAPGKGLEWVSGISNLGLTTGYADSVKGRFTISRDNSKNTLYLQMNSLRAEDTAVYYCAKTTSRFDYWGQGTLVTVSSASTKGPSVFPLAPCSRSTSESTAALGCLVKDYFPEPVTVSWNSGALTSGVHTFPAVLQSSGLYSLSSVVTVPSSSLGTKTYTCNVDHKPSNTKVDKRVESKYGPPCPPCPAPEAEKGPSVFLFPPKPKDTLYITREPEVTCVVVDVSQEDPEVQFNWYVDGVEVHNAKTKPREEQFNSTYRVVSVLTVLHQDWLNGKEYKCKVSNKGLPSSIEKTISKAKGQPREPQVYTLPPSQEEMTKNQVSLTCLVKGFYPSDIAVEWESNGQPENNYKTTPPVLDSDGSFFLYSRLTVDKSRWQEGNVFSCSVMHEALHNHYTQKSLSLSLGK

SEQ ID NO: 21 - protein, 443 aa, synthetic construct
EVQLLESGGGLVQPGGSLRLSCAASGFTFSSYAMSWVRQAPGKGLEWVSGISNLGLTTGYADSVKGRFTISRDNSKNTLYLQMNSLRAEDTAVYYCAKTTSRFDYWGQGTLVTVSSASTKGPSVFPLAPCSRSTSESTAALGCLVKDYFPEPVTVSWNSGALTSGVHTFPAVLQSSGLYSLSSVVTVPSSSLGTKTYTCNVDHKPSNTKVDKRVESKYGPPCPPCPAPEFEGGPSVFLFPPKPKDTLYITREPEVTCVVVDVSQEDPEVQFNWYVDGVEVHNAKTKPREEQFNSTYRVVSVLTVLHQDWLNGKEYKCKVSNKGLPSSIEKTISKAKGQPREPQVYTLPPSQEEMTKNQVSLTCLVKGFYPSDIAVEWESNGQPENNYKTTPPVLDSDGSFFLYSRLTVDKSRWQEGNVFSCSVMHEALHNHYTQKSLSLSLGK

SEQ ID NO: 22 - protein, 107 aa, synthetic construct [sequence omitted]

SEQ ID NO: 23 - protein, 327 aa, synthetic construct
ASTKGPSVFPLAPCSRSTSESTAALGCLVKDYFPEPVTVSWNSGALTSGVHTFPAVLQSSGLYSLSSVVTVPSSSLGTKTYTCNVDHKPSNTKVDKRVESKYGPPCPPCPAPEFEGGPSVFLFPPKPKDTLYITREPEVTCVVVDVSQEDPEVQFNWYVDGVEVHNAKTKPREEQFNSTYRVVSVLTVLHQDWLNGKEYKCKVSNKGLGSSIEKTISKAKGQPREPQVYTLPPSQEEMTKNQVSLTCLVKGFYPSDIAVEWESNGQPENNYKTTPPVLDSDGSFFLYSRLTVDKSRWQEGNVFSCSVMHEALHNHYTQKSLSLSLGK

SEQ ID NO: 24 - protein, 327 aa, synthetic construct
ASTKGPSVFPLAPCSRSTSESTAALGCLVKDYFPEPVTVSWNSGALTSGVHTFPAVLQSSGLYSLSSVVTVPSSSLGTKTYTCNVDHKPSNTKVDKRVESKYGPPCPPCPAPEAEGGPSVFLFPPKPKDTLYITREPEVTCVVVDVSQEDPEVQFNWYVDGVEVHNAKTKPREEQFNSTYRVVSVLTVLHQDWLNGKEYKCKVSNKGLPSSIEKTISKAKGQPREPQVYTLPPSQEEMTKNQVSLTCLVKGFYPSDIAVEWESNGQPENNYKTTPPVLDSDGSFFLYSKLTVDKSRWQEGNVFSCSVMHEALHNHYTQKSLSLSLGK

SEQ ID NO: 25 - protein, 327 aa, synthetic construct
ASTKGPSVFPLAPCSRSTSESTAALGCLVKDYFPEPVTVSWNSGALTSGVHTFPAVLQSSGLYSLSSVVTVPSSSLGTKTYTCNVDHKPSNTKVDKRVESKYGPPCPPCPAPEAEKGPSVFLFPPKPKDTLYITREPEVTCVVVDVSQEDPEVQFNWYVDGVEVHNAKTKPREEQFNSTYRVVSVLTVLHQDWLNGKEYKCKVSNKGLPSSIEKTISKAKGQPREPQVYTLPPSQEEMTKNQVSLTCLVKGFYPSDIAVEWESNGQPENNYKTTPPVLDSDGSFFLYSRLTVDKSRWQEGNVFSCSVMHEALHNHYTQKSLSLSLGK

SEQ ID NO: 26 - protein, 327 aa, synthetic construct
ASTKGPSVFPLAPCSRSTSESTAALGCLVKDYFPEPVTVSWNSGALTSGVHTFPAVLQSSGLYSLSSVVTVPSSSLGTKTYTCNVDHKPSNTKVDKRVESKYGPPCPPCPAPEFEGGPSVFLFPPKPKDTLYITREPEVTCVVVDVSQEDPEVQFNWYVDGVEVHNAKTKPREEQFNSTYRVVSVLTVLHQDWLNGKEYKCKVSNKGLPSSIEKTISKAKGQPREPQVYTLPPSQEEMTKNQVSLTCLVKGFYPSDIAVEWESNGQPENNYKTTPPVLDSDGSFFLYSRLTVDKSRWQEGNVFSCSVMHEALHNHYTQKSLSLSLGK

SEQ ID NO: 27 - protein, 242 aa, synthetic construct
MAEVQLLESGGGLVQPGGSLRLSCAASGFTFSSYAMSWVRQAPGKGLEWVSGISNLGLTTGYADSVKGRFTISRDNSKNTLYLQMNSLRAEDTAVYYCARTTSRFDYWGQGTLVTVSSGGGGSGGGGSGGGGSTDIQMTQSPSSLSASVGDRVTITCRASQSISSYLNWYQQKPGKAPKLLIYKASYLQSGVPSRFSGSGSGTDFTLTISSLQPEDFATYYCQNSAVRPVTFGQGTKVEIKR

SEQ ID NO: 28 - protein, 8 aa, synthetic construct
GFTFSSYA

SEQ ID NO: 29 - protein, 8 aa, synthetic construct
ISNLGLTT

SEQ ID NO: 30 - protein, 9 aa, synthetic construct
AKTTSRFDY

SEQ ID NO: 31 - protein, 6 aa, synthetic construct
QSISSY

SEQ ID NO: 32 - protein, 9 aa, synthetic construct
QNSAVRPVT

SEQ ID NO: 33 - protein, 443 aa, synthetic construct
EVQLLESGGGLVQPGGSLRLSCAASGFTFSSYAMSWVRQAPGKGLEWVSGISNLGLTTGYADSVKGRFTISRDNSKNTLYLQMNSLRAEDTAVYYCARTTSRFDYWGQGTLVTVSSASTKGPSVFPLAPCSRSTSESTAALGCLVKDYFPEPVTVSWNSGALTSGVHTFPAVLQSSGLYSLSSVVTVPSSSLGTKTYTCNVDHKPSNTKVDKRVESKYGPPCPPCPAPEFEGGPSVFLFPPKPKDTLYITREPEVTCVVVDVSQEDPEVQFNWYVDGVEVHNAKTKPREEQFNSTYRVVSVLTVLHQDWLNGKEYKCKVSNKGLGSSIEKTISKAKGQPREPQVYTLPPSQEEMTKNQVSLTCLVKGFYPSDIAVEWESNGQPENNYKTTPPVLDSDGSFFLYSRLTVDKSRWQEGNVFSCSVMHEALHNHYTQKSLSLSLGK

SEQ ID NO: 34 - protein, 443 aa, synthetic construct
EVQLLESGGGLVQPGGSLRLSCAASGFTFSSYAMSWVRQAPGKGLEWVSGISNLGLTTGYADSVKGRFTISRDNSKNTLYLQMNSLRAEDTAVYYCARTTSRFDYWGQGTLVTVSSASTKGPSVFPLAPCSRSTSESTAALGCLVKDYFPEPVTVSWNSGALTSGVHTFPAVLQSSGLYSLSSVVTVPSSSLGTKTYTCNVDHKPSNTKVDKRVESKYGPPCPPCPAPEAEGGPSVFLFPPKPKDTLYITREPEVTCVVVDVSQEDPEVQFNWYVDGVEVHNAKTKPREEQFNSTYRVVSVLTVLHQDWLNGKEYKCKVSNKGLPSSIEKTISKAKGQPREPQVYTLPPSQEEMTKNQVSLTCLVKGFYPSDIAVEWESNGQPENNYKTTPPVLDSDGSFFLYSKLTVDKSRWQEGNVFSCSVMHEALHNHYTQKSLSLSLGK

SEQ ID NO: 35 - protein, 443 aa, synthetic construct
EVQLLESGGGLVQPGGSLRLSCAASGFTFSSYAMSWVRQAPGKGLEWVSGISNLGLTTGYADSVKGRFTISRDNSKNTLYLQMNSLRAEDTAVYYCARTTSRFDYWGQGTLVTVSSASTKGPSVFPLAPCSRSTSESTAALGCLVKDYFPEPVTVSWNSGALTSGVHTFPAVLQSSGLYSLSSVVTVPSSSLGTKTYTCNVDHKPSNTKVDKRVESKYGPPCPPCPAPEAEKGPSVFLFPPKPKDTLYITREPEVTCVVVDVSQEDPEVQFNWYVDGVEVHNAKTKPREEQFNSTYRVVSVLTVLHQDWLNGKEYKCKVSNKGLPSSIEKTISKAKGQPREPQVYTLPPSQEEMTKNQVSLTCLVKGFYPSDIAVEWESNGQPENNYKTTPPVLDSDGSFFLYSRLTVDKSRWQEGNVFSCSVMHEALHNHYTQKSLSLSLGK

SEQ ID NO: 36 - protein, 443 aa, synthetic construct
EVQLLESGGGLVQPGGSLRLSCAASGFTFSSYAMSWVRQAPGKGLEWVSGISNLGLTTGYADSVKGRFTISRDNSKNTLYLQMNSLRAEDTAVYYCARTTSRFDYWGQGTLVTVSSASTKGPSVFPLAPCSRSTSESTAALGCLVKDYFPEPVTVSWNSGALTSGVHTFPAVLQSSGLYSLSSVVTVPSSSLGTKTYTCNVDHKPSNTKVDKRVESKYGPPCPPCPAPEFEGGPSVFLFPPKPKDTLYITREPEVTCVVVDVSQEDPEVQFNWYVDGVEVHNAKTKPREEQFNSTYRVVSVLTVLHQDWLNGKEYKCKVSNKGLPSSIEKTISKAKGQPREPQVYTLPPSQEEMTKNQVSLTCLVKGFYPSDIAVEWESNGQPENNYKTTPPVLDSDGSFFLYSRLTVDKSRWQEGNVFSCSVMHEALHNHYTQKSLSLSLGK